European Patent Specification EP 3 110 949 B1, published January 1, 2025. Title: MMP-8 activation product, its determination and use. Applicant: Oy Medix Biochemica Ab dentognostics GmbH. The sequence listing filed with the application follows.

SEQUENCE LISTING (2 sequences)

SEQ ID NO: 1 - protein, 14 aa, Homo sapiens
  peptide (1)..(14): amino acids 119-132
NYTPQLSEAEVERA

SEQ ID NO: 2 - protein, 16 aa, Homo sapiens
  peptide (1)..(16): amino acids 151-165
ISQGEADINIAFYQRD